European Patent Specification EP 3 359 576 B1, published December 25, 2024. Title: ANTIGEN-BINDING POLYPEPTIDE CONSTRUCTS COMPRISING KAPPA AND LAMBDA LIGHT CHAINS AND USES THEREOF. Applicant: Zymeworks Inc. Application NOT YET ASSIGNED. The sequence listing filed with the application follows.

SEQUENCE LISTING (20 sequences)

SEQ ID NO: 1 - protein, 227 aa, Artificial Sequence
  synthetic Pertuzumab heavy chain Fab (Domain boundaries: VH; E1 - S119, CH1; A120 - V217, Hinge (partial); E218 - T227)
EVQLVESGGGLVQPGGSLRLSCAASGFTFTDYTMDWVRQAPGKGLEWVADVNPNSGGSIYNQRFKGRFTLSVDRSKNTLYLQMNSLRAEDTAVYYCARNLGPSFYFDYWGQGTLVTVSSASTKGPSVFPLAPSSKSTSGGTAALGCLVKDYFPEPVTVSWNSGALTSGVHTFPAVLQSSGLYSLSSVVTVPSSSLGTQTYICNVNHKPSNTKVDKKVEPKSCDKTHT

SEQ ID NO: 2 - protein, 214 aa, Artificial Sequence
  synthetic Pertuzumab light chain (kappa) (Domain boundaries: VL; D1 - K107, CL; R108 - C214)
DIQMTQSPSSLSASVGDRVTITCKASQDVSIGVAWYQQKPGKAPKLLIYSASYRYTGVPSRFSGSGSGTDFTLTISSLQPEDFATYYCQQYYIYPYTFGQGTKVEIKRTVAAPSVFIFPPSDEQLKSGTASVVCLLNNFYPREAKVQWKVDNALQSGNSQESVTEQDSKDSTYSLSSTLTLSKADYEKHKVYACEVTHQGLSSPVTKSFNRGEC

SEQ ID NO: 3 - protein, 226 aa, Artificial Sequence
  synthetic CAT-2200 heavy chain Fab (Domain boundaries: VH; E1 - S118, CH1; A119 - V216, Hinge(partial); E217 - T226)
EVQLLESGGGLVQPGGSLRLSCAASGFTFSSYAMSWVRQAPGKGLEWVSAISGSGGSTYYADSVKGRFTISRDNSKNTLYLQMNSLRAEDTAVYYCARDLIHGVTRNWGQGTLVTVSSASTKGPSVFPLAPSSKSTSGGTAALGCLVKDYFPQPVTVSWNSGALTSGVHTFPAVLQSSGLYSLSSVVTVPSSSLGTQTYICNVNHKPSNTKVDKKVEPKSCDKTHT

SEQ ID NO: 4 - protein, 216 aa, Artificial Sequence
  synthetic CAT-2200 light chain (lambda) (Domain boundaries: VL; N1 - L110, CL; G111 - S216)
NFMLTQPHSVSESPGKTVTISCTRSSGSLANYYVQWYQQRPGSSPTIVIFANNQRPSGVPDRFSGSIDSSSNSASLTISGLKTEDEADYYCQTYDPYSVVFGGGTKLTVLGQPKAAPSVTLFPPSSEELQANKATLVCLISDFYPGAVTVAWKADSSPVKAGVETTTPSKQSNNKYAASSYLSLTPEQWKSHRSYSCQVTHEGSTVEKTVAPTECS

SEQ ID NO: 5 - protein, 222 aa, Artificial Sequence
  synthetic IgG1 Fc (Domain boundaries: Hinge (partial); C1 - P5, CH2; A6 - K115, CH3; G116 - K222)
CPPCPAPELLGGPSVFLFPPKPKDTLMISRTPEVTCVVVDVSHEDPEVKFNWYVDGVEVHNAKTKPREEQYNSTYRVVSVLTVLHQDWLNGKEYKCKVSNKALPAPIEKTISKAKGQPREPQVYTLPPSRDELTKNQVSLTCLVKGFYPSDIAVEWESNGQPENNYKTTPPVLDSDGSFFLYSKLTVDKSRWQQGNVFSCSVMHEALHNHYTQKSLSLSPGK

SEQ ID NO: 6 - DNA, 666 bp, Artificial Sequence
  synthetic IgG1 Fc
tgccctccctgtccagctccagaactgctgggaggacctagcgtgttcctgtttccccctaagccaaaagacactctgatgatttccaggactcccgaggtgacctgcgtggtggtggacgtgtctcacgaggaccccgaagtgaagttcaactggtacgtggatggcgtggaagtgcataatgctaagacaaaaccaagagaggaacagtacaactccacttatcgcgtcgtgagcgtgctgaccgtgctgcaccaggactggctgaacgggaaggagtataagtgcaaagtcagtaataaggccctgcctgctccaatcgaaaaaaccatctctaaggccaaaggccagccaagggagccccaggtgtacacactgccacccagcagagacgaactgaccaagaaccaggtgtccctgacatgtctggtgaaaggcttctatcctagtgatattgctgtggagtgggaatcaaatggacagccagagaacaattacaagaccacacctccagtgctggacagcgatggcagcttcttcctgtattccaagctgacagtggataaatctcgatggcagcaggggaacgtgtttagttgttcagtgatgcatgaagccctgcacaatcattacactcagaagagcctgtccctgtctcccggcaaa

SEQ ID NO: 7 - DNA, 681 bp, Artificial Sequence
  synthetic Pertuzumab heavy chain Fab
gaagtgcagctggtcgaatctggaggaggactggtgcagccaggagggtccctgcgcctgtcttgcgccgctagtggcttcacttttaccgactacaccatggattgggtgcgacaggcacctggaaagggcctggagtgggtcgccgatgtgaacccaaatagcggaggctccatctacaaccagcggttcaagggccggttcaccctgtcagtggaccggagcaaaaacaccctgtatctgcagatgaatagcctgcgagccgaagatactgctgtgtactattgcgcccggaatctggggccctccttctactttgactattgggggcagggaactctggtcaccgtgagctccgcctccaccaagggaccttctgtgttcccactggctccctctagtaaatccacatctgggggaactgcagccctgggctgtctggtgaaggactacttcccagagcccgtcacagtgtcttggaacagtggcgctctgacttctggggtccacacctttcctgcagtgctgcagtcaagcgggctgtacagcctgtcctctgtggtcaccgtgccaagttcaagcctgggaacacagacttatatctgcaacgtgaatcacaagccatccaatacaaaagtcgacaagaaagtggaacccaagtcttgtgataaaacccataca

SEQ ID NO: 8 - DNA, 642 bp, Artificial Sequence
  synthetic Pertuzumab light chain (kappa)
gatattcagatgacccagtccccaagctccctgagtgcctcagtgggcgaccgagtcaccatcacatgcaaggcttcccaggatgtgtctattggagtcgcatggtaccagcagaagccaggcaaagcacccaagctgctgatctatagcgcctcctaccggtataccggcgtgccctctagattctctggcagtgggtcaggaacagactttactctgaccatctctagtctgcagcctgaggatttcgctacctactattgccagcagtactatatctacccatatacctttggccaggggacaaaagtggagatcaagaggactgtggccgctccctccgtcttcatttttcccccttctgacgaacagctgaaaagtggcacagccagcgtggtctgtctgctgaacaatttctaccctcgcgaagccaaagtgcagtggaaggtcgataacgctctgcagagcggcaacagccaggagtctgtgactgaacaggacagtaaagattcaacctatagcctgtcaagcacactgactctgagcaaggcagactacgagaagcacaaagtgtatgcctgcgaagtcacacatcaggggctgtcctctcctgtgactaagagctttaacagaggagagtgt

SEQ ID NO: 9 - DNA, 678 bp, Artificial Sequence
  synthetic CAT-2200 heavy chain Fab
gaggtgcagctgctggaatctggggggggcctggtgcagcctggggggtccctgagactgtcatgtgctgccagcgggtttactttcagctcctacgctatgtcctgggtgcgacaggcacccgggaagggactggagtgggtctctgcaatcagtgggtcaggcgggagtacttactatgccgacagcgtgaagggacggttcactatctcaagagataacagcaagaacaccctgtatctgcagatgaacagcctgagagcagaagacacagccgtgtactattgcgccagggatctgatccacggagtcactcgcaattggggccaggggactctggtgaccgtctctagtgctagcacaaaggggccctctgtgtttccactggccccctcaagcaaaagcacatccggaggaactgcagctctgggatgtctggtgaaggactacttcccccagcctgtgaccgtctcttggaacagtggagccctgaccagcggcgtgcacacatttcctgctgtcctgcagtcctctggcctgtactccctgagttcagtggtcacagtgcctagctcctctctggggacccagacatatatttgcaacgtgaatcataaaccaagcaacactaaggtcgacaagaaagtggagcccaagagctgtgataaaactcatacc

SEQ ID NO: 10 - DNA, 648 bp, Artificial Sequence
  synthetic CAT-2200 light chain (lambda)
aactttatgctgactcagccccactccgtgtccgagagccctggcaaaactgtgactatttcatgtacccgatcatctggaagcctggccaactactatgtgcagtggtaccagcagaggccaggcagctcccccactatcgtgattttcgctaacaatcagcggccttccggcgtcccagacagattttccgggtctatcgattctagttcaaatagtgcatcactgactatttccgggctgaagaccgaggacgaagccgattactattgccagacctacgacccctattctgtggtcttcggcgggggaaccaagctgacagtgctgggacagccaaaagcggcgcccagtgtcacactgtttccccctagctccgaggaactgcaggctaacaaagcaacactggtgtgtctgatcagcgacttctaccctggagctgtgactgtcgcctggaaggctgattctagtccagtgaaagcaggcgtcgagaccacaactccctctaagcagagtaacaacaagtacgcagcctcaagctatctgtcactgaccccagaacagtggaagagccaccggagctattcctgccaggtcactcacgaaggctccactgtcgagaaaaccgtcgctcccaccgaatgttca

SEQ ID NO: 11 - protein, 217 aa, Artificial Sequence
  synthetic Human IgG1 Fc sequence 231-447 (EU-numbering), without hinge
APELLGGPSVFLFPPKPKDTLMISRTPEVTCVVVDVSHEDPEVKFNWYVDGVEVHNAKTKPREEQYNSTYRVVSVLTVLHQDWLNGKEYKCKVSNKALPAPIEKTISKAKGQPREPQVYTLPPSRDELTKNQVSLTCLVKGFYPSDIAVEWESNGQPENNYKTTPPVLDSDGSFFLYSKLTVDKSRWQQGNVFSCSVMHEALHNHYTQKSLSLSPGK

SEQ ID NO: 12 - protein, 228 aa, Artificial Sequence
  synthetic SGN-CD19a heavy chain Fab (Domain boundaries: VH; Q1-S120, CH1; A121-V218, Hinge (partial); E219-T228)
QVTLRESGPALVKPTQTLTLTCTFSGFSLSTSGMGVGWIRQPPGKALEWLAHIWWDDDKRYNPALKSRLTISKDTSKNQVVLTMTNMDPVDTAAYYCARMELWSYYFDYWGQGTLVTVSSASTKGPSVFPLAPSSKSTSGGTAALGCLVKDYFPEPVTVSWNSGALTSGVHTFPAVLQSSGLYSLSSVVTVPSSSLGTQTYICNVNHKPSNTKVDKKVEPKSCDKTHT

SEQ ID NO: 13 - protein, 213 aa, Artificial Sequence
  synthetic SGN-CD19a light chain (kappa) (Domain boundaries: VL; E1-K106, CL; R107-C213)
EIVLTQSPATLSLSPGERATLSCSASSSVSYMHWYQQKPGQAPRLLIYDTSKLASGIPARFSGSGSGTDFTLTISSLEPEDFAVYYCFQGSVYPFTFGQGTKLEIKRTVAAPSVFIFPPSDEQLKSGTASVVCLLNNFYPREAKVQWKVDNALQSGNSQESVTEQDSKDSTYSLSSTLTLSKADYEKHKVYACEVTHQGLSSPVTKSFNRGEC

SEQ ID NO: 14 - protein, 233 aa, Artificial Sequence
  synthetic CR8071 heavy chain Fab (Domain boundaries: VH; Q1-S125, CH1; A126-V223, Hinge (partial); E224-T233)
QVQLVQSGAEVKKPGASVRVSCRASGYIFTESGITWVRQAPGQGLEWMGWISGYSGDTKYAQKLQGRVTMTKDTSTTTAYMELRSLRYDDTAVYYCARDVQYSGSYLGAYYFDYWSPGTLVTVSSASTKGPSVFPLAPSSKSTSGGTAALGCLVKDYFPEPVTVSWNSGALTSGVHTFPAVLQSSGLYSLSSVVTVPSSSLGTQTYICNVNHKPSNTKVDKKVEPKSCDKTHT

SEQ ID NO: 15 - protein, 216 aa, Artificial Sequence
  synthetic CR8071 light chain (lambda) (Domain boundaries: VL; Q1-L110, CL; R111-S216)
QSVLTQPPSASGTPGQRVTISCSGSSSNIGTNYVYWYQQFPGTAPKLLIYRSYQRPSGVPDRFSGSKSGSSASLAISGLQSEDEADYYCATWDDSLDGWVFGGGTKLTVLRQPKAAPSVTLFPPSSEELQANKATLVCLISDFYPGAVTVAWKADSSPVKAGVETTTPSKQSNNKYAASSYLSLTPEQWKSHRSYSCQVTHEGSTVEKTVAPTECS

SEQ ID NO: 16 - DNA, 684 bp, Artificial Sequence
  synthetic SGN-CD19a heavy chain Fab
caggtgacactgagagaatccggcccagccctggtgaagcccactcagaccctgacactgacttgcaccttctctgggttttccctgtctacaagtgggatgggagtgggatggatcaggcagccacctggaaaagccctggagtggctggctcacatttggtgggacgatgacaagcggtacaacccagcactgaaaagcagactgacaatcagcaaggatacttccaaaaaccaggtggtcctgacaatgactaatatggaccccgtggacacagccgcttactattgcgcccgcatggaactgtggagctactatttcgactactgggggcagggaacactggtcactgtgagctccgctagcactaaggggccttccgtgtttccactggctccctctagtaaatccacctctggaggcacagctgcactgggatgtctggtgaaggattacttccctgaaccagtcacagtgagttggaactcaggggctctgacaagtggagtccatacttttcccgcagtgctgcagtcaagcggactgtactccctgtcctctgtggtcaccgtgcctagttcaagcctgggcacccagacatatatctgcaacgtgaatcacaagccatcaaatacaaaagtcgacaagaaagtggagcccaagagctgtgataaaactcatacc

SEQ ID NO: 17 - DNA, 639 bp, Artificial Sequence
  synthetic SGN-CD19a light chain (kappa)
gagatcgtgctgacccagtctccagccacactgtctctgagcccaggagagagggccaccctgtcctgctctgccagctccagcgtgagctacatgcactggtatcagcagaagccaggacaggcccctaggctgctgatctacgacaccagcaagctggcctccggcatccccgcaagattcagcggctccggctctggcacagactttaccctgacaatcagctccctggagcctgaggatttcgccgtgtactattgttttcagggcagcgtgtatccattcacctttggccagggcacaaagctggagatcaagcggacagtggcggcgcccagtgtcttcatttttccccctagcgacgaacagctgaagtctgggacagccagtgtggtctgtctgctgaacaacttctaccctagagaggctaaagtgcagtggaaggtcgataacgcactgcagtccggaaattctcaggagagtgtgactgaacaggactcaaaagatagcacctattccctgtcaagcacactgactctgagcaaggccgactacgagaagcataaagtgtatgcttgtgaagtcacccaccaggggctgagttcaccagtcacaaaatcattcaacagaggggagtgc

SEQ ID NO: 18 - DNA, 699 bp, Artificial Sequence
  synthetic CR8071 heavy chain Fab
caggtgcagctggtccagtccggggctgaagtgaaaaaacctggggcatccgtgcgggtgtcatgtcgggcaagcgggtatatctttactgagtctggaatcacctgggtgaggcaggctcccggacagggactggaatggatgggatggatttctggatacagtggcgacacaaagtatgcacagaaactgcagggccgcgtcaccatgacaaaggatacttcaaccacaactgcctacatggagctgcggagcctgagatatgacgatacagccgtgtactattgcgcccgggacgtgcagtacagcgggtcctacctgggggcatactacttcgattactggtcacctggaactctggtcaccgtctcttcagctagcaccaagggcccttctgtgtttccactggcaccctcaagcaaaagcacctccggaggaacagcagcactgggatgtctggtcaaggactatttccccgagcctgtgaccgtctcatggaatagcggcgcactgactagtggggtgcacacctttcccgccgtcctgcagtcctctgggctgtacagcctgagttcagtggtcacagtgccaagctcctctctgggaactcagacctatatctgcaacgtcaatcataaacccagcaacacaaaggtcgacaagaaagtggagcccaagagctgtgataaaactcatacc

SEQ ID NO: 19 - DNA, 648 bp, Artificial Sequence
  synthetic CR8071 light chain (lambda)
cagagcgtcctgactcagcctccctccgcctccggaacacctgggcagagagtgactatctcctgtagcggatcaagctcaaacattggaaccaactacgtgtattggtaccagcagttccccggcacagctcctaagctgctgatctatcggagctaccagagaccaagcggggtccccgacaggttttctggcagtaaatcagggagctccgccagcctggctatttccggcctgcagtctgaggacgaagcagattactattgcgccacctgggacgattccctggatggatgggtcttcggcggcggcacaaaactgaccgtcctgaggcagccaaaggcggcgcccagtgtcacactgtttccccctagctccgaggaactgcaggctaacaaagcaacactggtgtgtctgatcagcgacttctaccctggagctgtgactgtcgcctggaaggctgattctagtccagtgaaagcaggcgtcgagaccacaactccctctaagcagagtaacaacaagtacgcagcctcaagctatctgtcactgaccccagaacagtggaagagccaccggagctattcctgccaggtcactcacgaaggctccactgtcgagaaaaccgtcgctcccaccgaatgttca

SEQ ID NO: 20 - protein, 217 aa, Artificial Sequence
  Synthetic variant Human IgG1 Fc sequence 231-447 (EU-numbering), without hinge
  MISC_FEATURE (120)..(120): Xaa is Thr or Val
  MISC_FEATURE (121)..(121): Xaa is Leu or Tyr
  MISC_FEATURE (136)..(136): Xaa is Thr or Leu
  MISC_FEATURE (160)..(160): Xaa is Asn or Arg
  MISC_FEATURE (162)..(162): Xaa is Lys, Met or Leu
  MISC_FEATURE (164)..(164): Xaa is Thr or Trp
  MISC_FEATURE (170)..(170): Xaa is Ser or Glu
  MISC_FEATURE (175)..(175): Xaa is Phe or Ala
  MISC_FEATURE (177)..(177): Xaa is Tyr or Val
APELLGGPSVFLFPPKPKDTLMISRTPEVTCVVVDVSHEDPEVKFNWYVDGVEVHNAKTKPREEQYNSTYRVVSVLTVLHQDWLNGKEYKCKVSNKALPAPIEKTISKAKGQPREPQVYXXPPSRDELTKNQVSLXCLVKGFYPSDIAVEWESNGQPENXYXTXPPVLDXDGSFXLXSKLTVDKSRWQQGNVFSCSVMHEALHNHYTQKSLSLSPGK